European Patent Application EP 4 129 338 A1, published February 8, 2023. Title: Treatment or prevention of aneurysm by using miR-33b inhibitor. Applicant: Mitsubishi Tanabe Pharma Corporation Kyoto University Osaka University National Institutes of Biomedical Innovation, Health and Nutrition. The sequence listing filed with the application follows.

SEQUENCE LISTING (23 sequences)

SEQ ID NO: 1 - RNA, 20 nt, Homo sapiens
gugcauugcuguugcauugc

SEQ ID NO: 2 - RNA, 21 nt, Homo sapiens
gugcauuguaguugcauugca

SEQ ID NO: 3 - RNA, 21 nt, Homo sapiens
gugcauuguaguugcauugca

SEQ ID NO: 4 - RNA, 96 nt, Homo sapiens
gcgggcggccccgcggugcauugcuguugcauugcacgugugugaggcgggugcagugccucggcagugcagcccggagccggccccuggcaccac

SEQ ID NO: 5 - DNA, 12 bp, Artificial Sequence
  antisense oligonucleotide
aacagcaatgca

SEQ ID NO: 6 - DNA, 16 bp, Artificial Sequence
  antisense oligonucleotide
tgcaacagcaatgcac

SEQ ID NO: 7 - DNA, 12 bp, Artificial Sequence
  antisense oligonucleotide
  modified_base (3)..(3): m5c
  modified_base (11)..(11): m5c
aactacaatgca

SEQ ID NO: 8 - DNA, 12 bp, Artificial Sequence
  antisense oligonucleotide
  modified_base (3)..(3): m5c
  modified_base (11)..(11): m5c
aacagcaatgca

SEQ ID NO: 9 - DNA, 16 bp, Artificial Sequence
  antisense oligonucleotide
  modified_base (3)..(3): m5c
  modified_base (9)..(9): m5c
tgcaactacaatgcac

SEQ ID NO: 10 - DNA, 16 bp, Artificial Sequence
  antisense oligonucleotide
  modified_base (3)..(3): m5c
  modified_base (9)..(9): m5c
tgcaacagcaatgcac

SEQ ID NO: 11 - DNA, 12 bp, Artificial Sequence
  antisense oligonucleotide
  modified_base (3)..(3): m5c
  modified_base (11)..(11): m5c
aacaatactacg

SEQ ID NO: 12 - DNA, 22 bp, Artificial Sequence
  primer
aacagtcccactggtcgtagat

SEQ ID NO: 13 - DNA, 22 bp, Artificial Sequence
  primer
tgttgcagaaagcgaatgtagt

SEQ ID NO: 14 - DNA, 20 bp, Artificial Sequence
  primer
aggcactcttccagccttcc

SEQ ID NO: 15 - DNA, 20 bp, Artificial Sequence
  primer
gcactgtgttggcgtacagg

SEQ ID NO: 16 - DNA, 20 bp, Artificial Sequence
  primer
ttgacagcgacaagaagtgg

SEQ ID NO: 17 - DNA, 20 bp, Artificial Sequence
  primer
gccattcacgtcgtccttat

SEQ ID NO: 18 - DNA, 20 bp, Artificial Sequence
  primer
ccccagtcacctgctgttat

SEQ ID NO: 19 - DNA, 20 bp, Artificial Sequence
  primer
tggaatcctgaacccacttc

SEQ ID NO: 20 - DNA, 20 bp, Artificial Sequence
  primer
tgcctgactcacactcaagg

SEQ ID NO: 21 - DNA, 20 bp, Artificial Sequence
  primer
ggcttctcagcaactgaacc

SEQ ID NO: 22 - DNA, 20 bp, Artificial Sequence
  primer
aacagtttgtggcccttttg

SEQ ID NO: 23 - DNA, 20 bp, Artificial Sequence
  primer
agttccaggctggggtactt